European Patent Specification EP 3 634 474 B1, published May 6, 2026. Title: Targeting modules for universal chimeric antigen receptor expressing immune cells and use in the treatment of cancer, infections and autoimmune disorders. Applicant: GEMoaB Monoclonals GmbH. The sequence listing filed with the application follows.

SEQUENCE LISTING (27 sequences)

SEQ ID NO: 1 - DNA, 1806 bp, Artificial Sequence
  Homo sapiens/Mus musculus chimera
atgcgccgcatgcagctgctgcttctgatcgctctgagcctggctcttgtgaccaactctgaattccaggtgcagctggtgcagagcggagccgaggtgaagaagcctggagcctctgtgaaggtgagctgcaaggcttctggctacaccttcacccactactacatctactgggtgagacaggctcccggacagggcctggagtggatgggaggcgtgaaccccagcaacggaggcacccacttcaacgagaagttcaagtctcgcgtgaccatgacccgcgacaccagcatctctaccgcttacatggagctgagccgcctgcgctctgatgataccgctgtgtactactgcgctcgcagcgagtacgattacggactgggcttcgcctactggggccagggaaccctggtgaccgtgagctctggaggcggaggcagcggaggcggcggatctggaggcggaggaagcgatatcgtgatgacccagtctcctgatagcctggctgtgagcctgggcgagagagctaccatcaactgcaagagcagccagagcctgctgaactctcgcacccctaagaactaccttgcttggtaccagcagaagcctggacagccccctaagctgctgatctactgggcttctacccgcaagagcggcgtgcccgacagattctctggcagcggaagcggcaccgatttcaccctgaccatcagcagcctgcaggctgaggacgtggccgtgtactactgcaagcagtcttacaacctgctgaccttcggaggcggaaccaaggtggagatcaaggctgccgctggaggaggcggcagcaagatcctggtcaaacagtcccctatgctggtcgcttacgacaacgccgttaatctgagttgcaaatatagttacaacctgtttagccgggaatttcgcgcatctctccacaagggactggattctgcggttgaggtttgtgtggtctatggcaattatagccagcaactgcaagtgtacagcaaaacaggctttaactgcgacgggaaactcgggaacgaatcagtgaccttctatctgcagaacctgtacgttaaccaaacagatatttacttctgcaagatagaggtgatggctccaccgccagcactggataacgagaagtccaatggaaccatcattcacgtcaaggggaagcatctgtgtccttccccgttgttccctgggccgagcaaacccttttgggtgcttgtggtagttggcggggtattggcctgctattcccttctcgtaactgtggccttcatcatcttctgggtcagatctaagaggtctaggggcgggcatagcgactacatgaacatgacacccaggcggcctggccccactcgcaaacactaccagccatacgcaccaccaagagactttgccgcatatcggagtggtggcggcgggtcaggaggtggagctagcggtggaggaggttccttctctaggtcagctgatgctcccgcctatcagcaaggtcagaaccagctctacaatgagctgaatctgggacgtcgggaggagtacgacgtgctggataaacgaagaggacgcgatcccgagatgggtgggaagcctaggcgcaagaatccccaggaaggcctctacaatgaactgcagaaagacaagatggccgaagcctacagcgagattggcatgaaaggggagcgacggagaggaaagggacatgacgggttgtatcagggtctttccactgcgacaaaggatacctatggggctctgcacatgcaagcactgccacctaga

SEQ ID NO: 2 - DNA, 60 bp, Homo sapiens
atgcgccgcatgcagctgctgcttctgatcgctctgagcctggctcttgtgaccaactct

SEQ ID NO: 3 - DNA, 360 bp, Artificial Sequence
  Homo sapiens/Mus musculus chimera
caggtgcagctggtgcagagcggagccgaggtgaagaagcctggagcctctgtgaaggtgagctgcaaggcttctggctacaccttcacccactactacatctactgggtgagacaggctcccggacagggcctggagtggatgggaggcgtgaaccccagcaacggaggcacccacttcaacgagaagttcaagtctcgcgtgaccatgacccgcgacaccagcatctctaccgcttacatggagctgagccgcctgcgctctgatgataccgctgtgtactactgcgctcgcagcgagtacgattacggactgggcttcgcctactggggccagggaaccctggtgaccgtgagctct

SEQ ID NO: 4 - DNA, 336 bp, Artificial Sequence
  Homo sapiens/Mus musculus chimera
gatatcgtgatgacccagtctcctgatagcctggctgtgagcctgggcgagagagctaccatcaactgcaagagcagccagagcctgctgaactctcgcacccctaagaactaccttgcttggtaccagcagaagcctggacagccccctaagctgctgatctactgggcttctacccgcaagagcggcgtgcccgacagattctctggcagcggaagcggcaccgatttcaccctgaccatcagcagcctgcaggctgaggacgtggccgtgtactactgcaagcagtcttacaacctgctgaccttcggaggcggaaccaaggtggagatcaag

SEQ ID NO: 5 - DNA, 399 bp, Homo sapiens
aagatcctggtcaaacagtcccctatgctggtcgcttacgacaacgccgttaatctgagttgcaaatatagttacaacctgtttagccgggaatttcgcgcatctctccacaagggactggattctgcggttgaggtttgtgtggtctatggcaattatagccagcaactgcaagtgtacagcaaaacaggctttaactgcgacgggaaactcgggaacgaatcagtgaccttctatctgcagaacctgtacgttaaccaaacagatatttacttctgcaagatagaggtgatggctccaccgccagcactggataacgagaagtccaatggaaccatcattcacgtcaaggggaagcatctgtgtccttccccgttgttccctgggccgagcaaaccc

SEQ ID NO: 6 - DNA, 81 bp, Homo sapiens
ttttgggtgcttgtggtagttggcggggtattggcctgctattcccttctcgtaactgtggccttcatcatcttctgggtc

SEQ ID NO: 7 - DNA, 123 bp, Homo sapiens
agatctaagaggtctaggggcgggcatagcgactacatgaacatgacacccaggcggcctggccccactcgcaaacactaccagccatacgcaccaccaagagactttgccgcatatcggagt

SEQ ID NO: 8 - DNA, 327 bp, Homo sapiens
ttctctaggtcagctgatgctcccgcctatcagcaaggtcagaaccagctctacaatgagctgaatctgggacgtcgggaggagtacgacgtgctggataaacgaagaggacgcgatcccgagatgggtgggaagcctaggcgcaagaatccccaggaaggcctctacaatgaactgcagaaagacaagatggccgaagcctacagcgagattggcatgaaaggggagcgacggagaggaaagggacatgacgggttgtatcagggtctttccactgcgacaaaggatacctatggggctctgcacatgcaagcactgccacctaga

SEQ ID NO: 9 - DNA, 1512 bp, Artificial Sequence
  Homo sapiens/Mus musculus chimera
atgcgccgcatgcagctgctgcttctgatcgctctgagcctggctcttgtgaccaactctgaattccaggtgcagctggtgcagagcggagccgaggtgaagaagcctggagcctctgtgaaggtgagctgcaaggcttctggctacaccttcacccactactacatctactgggtgagacaggctcccggacagggcctggagtggatgggaggcgtgaaccccagcaacggaggcacccacttcaacgagaagttcaagtctcgcgtgaccatgacccgcgacaccagcatctctaccgcttacatggagctgagccgcctgcgctctgatgataccgctgtgtactactgcgctcgcagcgagtacgattacggactgggcttcgcctactggggccagggaaccctggtgaccgtgagctctggaggcggaggcagcggaggcggcggatctggaggcggaggaagcgatatcgtgatgacccagtctcctgatagcctggctgtgagcctgggcgagagagctaccatcaactgcaagagcagccagagcctgctgaactctcgcacccctaagaactaccttgcttggtaccagcagaagcctggacagccccctaagctgctgatctactgggcttctacccgcaagagcggcgtgcccgacagattctctggcagcggaagcggcaccgatttcaccctgaccatcagcagcctgcaggctgaggacgtggccgtgtactactgcaagcagtcttacaacctgctgaccttcggaggcggaaccaaggtggagatcaagggaggaggcgggtcaaccactacccctgctcccaggcctcctacacccgcgccaacgattgccagtcaacctctgtccctgaggcctgaagcctgcagaccagctgcaggcggtgctgtgcatacacggggcttggactttgcctgcgatatctacatctgggcacctcttgccgggacttgtggcgttctcctgctttctctggtcattaccctgtactgtggaggcggcggtagcaaacgcggacggaagaaactgctgtacatcttcaagcagcccttcatgcgccccgtgcagacaacacaggaagaggacggttgcagctgccgatttcccgaagaggaggagggaggctgtgaattgggcggaggaggctccttctctcgcagtgcagatgccccagcgtacaagcaaggccagaaccagctgtacaacgagctcaatctggggcgtagagaggagtatgacgtgctggacaagaggcgaggaagggaccccgagatgggtggcaaaccgcggcgtaagaatccgcaggaaggcctctacaacgagctgcagaaagacaagatggccgaagcctattccgagatagggatgaaaggggaaagacggcgcggtaaagggcacgatgggctctatcagggtctgagcactgcaaccaaggacacgtatgatgccttgcacatgcaagctcttccaccaaga

SEQ ID NO: 10 - DNA, 135 bp, Homo sapiens
accactacccctgctcccaggcctcctacacccgcgccaacgattgccagtcaacctctgtccctgaggcctgaagcctgcagaccagctgcaggcggtgctgtgcatacacggggcttggactttgcctgcgat

SEQ ID NO: 11 - DNA, 72 bp, Homo sapiens
atctacatctgggcacctcttgccgggacttgtggcgttctcctgctttctctggtcattaccctgtactgt

SEQ ID NO: 12 - DNA, 126 bp, Homo sapiens
aaacgcggacggaagaaactgctgtacatcttcaagcagcccttcatgcgccccgtgcagacaacacaggaagaggacggttgcagctgccgatttcccgaagaggaggagggaggctgtgaattg

SEQ ID NO: 13 - DNA, 1806 bp, Artificial Sequence
  Homo sapiens/Mus musculus chimera
atgcgccgcatgcagctgctgcttctgatcgctctgagcctggctcttgtgaccaactctgaattccaggtggaggtgcaactggtcgaaagtggcggtggtttagttcagcctggtggaagtctacggcttagctgcgcagcatccggtttcacctttagcgacttttggatgaactgggttcggcaggctccgggcaaaggactggagtgggttgggcaaatccgcaacaaaccgaataactacgaaacttattactcagatagcctgaagggtcgattcaccatcagcagggatgattcaaagtcaatcacttacctacagatgaactcattaagagcggaggatactgcggtgtattactgtacactaggtaactcctggttcgcgtattggggacagggcacccttgtaaccgtctccagcggaggcggaggcagcggaggcggcggatctggaggcggaggaagcgacattgttatgacccagagcccggactctctcgctgttagtcttggtgagcgagcgactattaactgccggagcagtcagagtttgttggactctcggacgaaaaagaactacctggcatggtaccagcagaagccgggccaaccacctaaattactgatatattgggcgtcgactcgtgagtcaggggtaccggacaggttttctggaagcggatcaggaacagacttcactttgacgatctcttcgcttcaagccgaggacgttgcggtttattattgtaagcaaagctataatctgccgacatttggtggcggcaccaaggttgaaattaaggctgccgctggaggaggcggcagcaagatcctggtcaaacagtcccctatgctggtcgcttacgacaacgccgttaatctgagttgcaaatatagttacaacctgtttagccgggaatttcgcgcatctctccacaagggactggattctgcggttgaggtttgtgtggtctatggcaattatagccagcaactgcaagtgtacagcaaaacaggctttaactgcgacgggaaactcgggaacgaatcagtgaccttctatctgcagaacctgtacgttaaccaaacagatatttacttctgcaagatagaggtgatggctccaccgccagcactggataacgagaagtccaatggaaccatcattcacgtcaaggggaagcatctgtgtccttccccgttgttccctgggccgagcaaacccttttgggtgcttgtggtagttggcggggtattggcctgctattcccttctcgtaactgtggccttcatcatcttctgggtcagatctaagaggtctaggggcgggcatagcgactacatgaacatgacacccaggcggcctggccccactcgcaaacactaccagccatacgcaccaccaagagactttgccgcatatcggagtggtggcggcgggtcaggaggtggagctagcggtggaggaggttccttctctaggtcagctgatgctcccgcctatcagcaaggtcagaaccagctctacaatgagctgaatctgggacgtcgggaggagtacgacgtgctggataaacgaagaggacgcgatcccgagatgggtgggaagcctaggcgcaagaatccccaggaaggcctctacaatgaactgcagaaagacaagatggccgaagcctacagcgagattggcatgaaaggggagcgacggagaggaaagggacatgacgggttgtatcagggtctttccactgcgacaaaggatacctatggggctctgcacatgcaagcactgccacctaga

SEQ ID NO: 14 - DNA, 354 bp, Artificial Sequence
  Homo sapiens/Mus musculus chimera
gaggtgcaactggtcgaaagtggcggtggtttagttcagcctggtggaagtctacggcttagctgcgcagcatccggtttcacctttagcgacttttggatgaactgggttcggcaggctccgggcaaaggactggagtgggttgggcaaatccgcaacaaaccgaataactacgaaacttattactcagatagcctgaagggtcgattcaccatcagcagggatgattcaaagtcaatcacttacctacagatgaactcattaagagcggaggatactgcggtgtattactgtacactaggtaactcctggttcgcgtattggggacagggcacccttgtaaccgtctccagc

SEQ ID NO: 15 - DNA, 336 bp, Artificial Sequence
  Homo sapiens/Mus musculus chimera
gacattgttatgacccagagcccggactctctcgctgttagtcttggtgagcgagcgactattaactgccggagcagtcagagtttgttggactctcggacgaaaaagaactacctggcatggtaccagcagaagccgggccaaccacctaaattactgatatattgggcgtcgactcgtgagtcaggggtaccggacaggttttctggaagcggatcaggaacagacttcactttgacgatctcttcgcttcaagccgaggacgttgcggtttattattgtaagcaaagctataatctgccgacatttggtggcggcaccaaggttgaaattaag

SEQ ID NO: 16 - DNA, 1506 bp, Artificial Sequence
  Homo sapiens/Mus musculus chimera
atgcgccgcatgcagctgctgcttctgatcgctctgagcctggctcttgtgaccaactctgaattcgaggtgcaactggtcgaaagtggcggtggtttagttcagcctggtggaagtctacggcttagctgcgcagcatccggtttcacctttagcgacttttggatgaactgggttcggcaggctccgggcaaaggactggagtgggttgggcaaatccgcaacaaaccgaataactacgaaacttattactcagatagcctgaagggtcgattcaccatcagcagggatgattcaaagtcaatcacttacctacagatgaactcattaagagcggaggatactgcggtgtattactgtacactaggtaactcctggttcgcgtattggggacagggcacccttgtaaccgtctccagcggaggcggaggcagcggaggcggcggatctggaggcggaggaagcgacattgttatgacccagagcccggactctctcgctgttagtcttggtgagcgagcgactattaactgccggagcagtcagagtttgttggactctcggacgaaaaagaactacctggcatggtaccagcagaagccgggccaaccacctaaattactgatatattgggcgtcgactcgtgagtcaggggtaccggacaggttttctggaagcggatcaggaacagacttcactttgacgatctcttcgcttcaagccgaggacgttgcggtttattattgtaagcaaagctataatctgccgacatttggtggcggcaccaaggttgaaattaagggaggaggcgggtcaaccactacccctgctcccaggcctcctacacccgcgccaacgattgccagtcaacctctgtccctgaggcctgaagcctgcagaccagctgcaggcggtgctgtgcatacacggggcttggactttgcctgcgatatctacatctgggcacctcttgccgggacttgtggcgttctcctgctttctctggtcattaccctgtactgtggaggcggcggtagcaaacgcggacggaagaaactgctgtacatcttcaagcagcccttcatgcgccccgtgcagacaacacaggaagaggacggttgcagctgccgatttcccgaagaggaggagggaggctgtgaattgggcggaggaggctccttctctcgcagtgcagatgccccagcgtacaagcaaggccagaaccagctgtacaacgagctcaatctggggcgtagagaggagtatgacgtgctggacaagaggcgaggaagggaccccgagatgggtggcaaaccgcggcgtaagaatccgcaggaaggcctctacaacgagctgcagaaagacaagatggccgaagcctattccgagatagggatgaaaggggaaagacggcgcggtaaagggcacgatgggctctatcagggtctgagcactgcaaccaaggacacgtatgatgccttgcacatgcaagctcttccaccaaga

SEQ ID NO: 17 - protein, 602 aa, Artificial Sequence
  Homo sapiens/Mus musculus chimera
MRRMQLLLLIALSLALVTNSEFQVQLVQSGAEVKKPGASVKVSCKASGYTFTHYYIYWVRQAPGQGLEWMGGVNPSNGGTHFNEKFKSRVTMTRDTSISTAYMELSRLRSDDTAVYYCARSEYDYGLGFAYWGQGTLVTVSSGGGGSGGGGSGGGGSDIVMTQSPDSLAVSLGERATINCKSSQSLLNSRTPKNYLAWYQQKPGQPPKLLIYWASTRKSGVPDRFSGSGSGTDFTLTISSLQAEDVAVYYCKQSYNLLTFGGGTKVEIKAAAGGGGSKILVKQSPMLVAYDNAVNLSCKYSYNLFSREFRASLHKGLDSAVEVCVVYGNYSQQLQVYSKTGFNCDGKLGNESVTFYLQNLYVNQTDIYFCKIEVMAPPPALDNEKSNGTIIHVKGKHLCPSPLFPGPSKPFWVLVVVGGVLACYSLLVTVAFIIFWVRSKRSRGGHSDYMNMTPRRPGPTRKHYQPYAPPRDFAAYRSGGGGSGGGASGGGGSFSRSADAPAYQQGQNQLYNELNLGRREEYDVLDKRRGRDPEMGGKPRRKNPQEGLYNELQKDKMAEAYSEIGMKGERRRGKGHDGLYQGLSTATKDTYGALHMQALPPR

SEQ ID NO: 18 - protein, 504 aa, Artificial Sequence
  Homo sapiens/Mus musculus chimera
MRRMQLLLLIALSLALVTNSEFQVQLVQSGAEVKKPGASVKVSCKASGYTFTHYYIYWVRQAPGQGLEWMGGVNPSNGGTHFNEKFKSRVTMTRDTSISTAYMELSRLRSDDTAVYYCARSEYDYGLGFAYWGQGTLVTVSSGGGGSGGGGSGGGGSDIVMTQSPDSLAVSLGERATINCKSSQSLLNSRTPKNYLAWYQQKPGQPPKLLIYWASTRKSGVPDRFSGSGSGTDFTLTISSLQAEDVAVYYCKQSYNLLTFGGGTKVEIKGGGGSTTTPAPRPPTPAPTIASQPLSLRPEACRPAAGGAVHTRGLDFACDIYIWAPLAGTCGVLLLSLVITLYCGGGGSKRGRKKLLYIFKQPFMRPVQTTQEEDGCSCRFPEEEEGGCELGGGGSFSRSADAPAYKQGQNQLYNELNLGRREEYDVLDKRRGRDPEMGGKPRRKNPQEGLYNELQKDKMAEAYSEIGMKGERRRGKGHDGLYQGLSTATKDTYDALHMQALPPR

SEQ ID NO: 19 - protein, 602 aa, Artificial Sequence
  Homo sapiens/Mus musculus chimera
MRRMQLLLLIALSLALVTNSEFQVEVQLVESGGGLVQPGGSLRLSCAASGFTFSDFWMNWVRQAPGKGLEWVGQIRNKPNNYETYYSDSLKGRFTISRDDSKSITYLQMNSLRAEDTAVYYCTLGNSWFAYWGQGTLVTVSSGGGGSGGGGSGGGGSDIVMTQSPDSLAVSLGERATINCRSSQSLLDSRTKKNYLAWYQQKPGQPPKLLIYWASTRESGVPDRFSGSGSGTDFTLTISSLQAEDVAVYYCKQSYNLPTFGGGTKVEIKAAAGGGGSKILVKQSPMLVAYDNAVNLSCKYSYNLFSREFRASLHKGLDSAVEVCVVYGNYSQQLQVYSKTGFNCDGKLGNESVTFYLQNLYVNQTDIYFCKIEVMAPPPALDNEKSNGTIIHVKGKHLCPSPLFPGPSKPFWVLVVVGGVLACYSLLVTVAFIIFWVRSKRSRGGHSDYMNMTPRRPGPTRKHYQPYAPPRDFAAYRSGGGGSGGGASGGGGSFSRSADAPAYQQGQNQLYNELNLGRREEYDVLDKRRGRDPEMGGKPRRKNPQEGLYNELQKDKMAEAYSEIGMKGERRRGKGHDGLYQGLSTATKDTYGALHMQALPPR

SEQ ID NO: 20 - protein, 502 aa, Artificial Sequence
  Homo sapiens/Mus musculus chimera
MRRMQLLLLIALSLALVTNSEFEVQLVESGGGLVQPGGSLRLSCAASGFTFSDFWMNWVRQAPGKGLEWVGQIRNKPNNYETYYSDSLKGRFTISRDDSKSITYLQMNSLRAEDTAVYYCTLGNSWFAYWGQGTLVTVSSGGGGSGGGGSGGGGSDIVMTQSPDSLAVSLGERATINCRSSQSLLDSRTKKNYLAWYQQKPGQPPKLLIYWASTRESGVPDRFSGSGSGTDFTLTISSLQAEDVAVYYCKQSYNLPTFGGGTKVEIKGGGGSTTTPAPRPPTPAPTIASQPLSLRPEACRPAAGGAVHTRGLDFACDIYIWAPLAGTCGVLLLSLVITLYCGGGGSKRGRKKLLYIFKQPFMRPVQTTQEEDGCSCRFPEEEEGGCELGGGGSFSRSADAPAYKQGQNQLYNELNLGRREEYDVLDKRRGRDPEMGGKPRRKNPQEGLYNELQKDKMAEAYSEIGMKGERRRGKGHDGLYQGLSTATKDTYDALHMQALPPR

SEQ ID NO: 21 - protein, 120 aa, Artificial Sequence
  Homo sapiens/Mus musculus chimera
QVQLVQSGAEVKKPGASVKVSCKASGYTFTHYYIYWVRQAPGQGLEWMGGVNPSNGGTHFNEKFKSRVTMTRDTSISTAYMELSRLRSDDTAVYYCARSEYDYGLGFAYWGQGTLVTVSS

SEQ ID NO: 22 - protein, 112 aa, Artificial Sequence
  Homo sapiens/Mus musculus chimera
DIVMTQSPDSLAVSLGERATINCKSSQSLLNSRTPKNYLAWYQQKPGQPPKLLIYWASTRKSGVPDRFSGSGSGTDFTLTISSLQAEDVAVYYCKQSYNLLTFGGGTKVEIK

SEQ ID NO: 23 - protein, 118 aa, Artificial Sequence
  Homo sapiens/Mus musculus chimera
EVQLVESGGGLVQPGGSLRLSCAASGFTFSDFWMNWVRQAPGKGLEWVGQIRNKPNNYETYYSDSLKGRFTISRDDSKSITYLQMNSLRAEDTAVYYCTLGNSWFAYWGQGTLVTVSS

SEQ ID NO: 24 - protein, 112 aa, Artificial Sequence
  Homo sapiens/Mus musculus chimera
DIVMTQSPDSLAVSLGERATINCRSSQSLLDSRTKKNYLAWYQQKPGQPPKLLIYWASTRESGVPDRFSGSGSGTDFTLTISSLQAEDVAVYYCKQSYNLPTFGGGTKVEIK

SEQ ID NO: 25 - protein, 10 aa, Homo sapiens
KPLPEVTDEY

SEQ ID NO: 26 - protein, 48 aa, Artificial Sequence
  Homo sapiens
CGEMGWVRCGGGGSGGGGSKPLPEVTDEYGGGGSGGGGSCGEMGWVRC

SEQ ID NO: 27 - protein, 18 aa, Homo sapiens
EKEALKKIIEDQQESLNK